European Patent Specification EP 3 668 531 B1, published June 24, 2026. Title: METHODS FOR TREATING AND/OR PREVENTING GRAFT-VERSUS-HOST DISEASE AND/OR DIFFUSE ALVEOLAR HEMORRHAGE AND/OR VENO-OCCLUSIVE DISEASE ASSOCIATED WITH HEMATOPOIETIC STEM CELL TRANSPLANT. Applicant: Omeros Corporation University of Leicester Demopulos, Gregory A. Dudler, Thomas Schwaeble, Hans-Wilhelm. The sequence listing filed with the application follows.

SEQUENCE LISTING (71 sequences)

SEQ ID NO: 1 - DNA, 725 bp, Homo sapiens
  CDS (27)..(584)
ggccaggccagctggacgggcacaccatgaggctgctgaccctcctgggccttctgtgtggctcggtggccacccccttgggcccgaagtggcctgaacctgtgttcgggcgcctggcatcccccggctttccaggggagtatgccaatgaccaggagcggcgctggaccctgactgcaccccccggctaccgcctgcgcctctacttcacccacttcgacctggagctctcccacctctgcgagtacgacttcgtcaagctgagctcgggggccaaggtgctggccacgctgtgcgggcaggagagcacagacacggagcgggcccctggcaaggacactttctactcgctgggctccagcctggacattaccttccgctccgactactccaacgagaagccgttcacggggttcgaggccttctatgcagccgaggacattgacgagtgccaggtggccccgggagaggcgcccacctgcgaccaccactgccacaaccacctgggcggtttctactgctcctgccgcgcaggctacgtcctgcaccgtaacaagcgcacctgctcagagcagagcctctagcctcccctggagctccggcctgcccagcaggtcagaagccagagccagcctgctggcctcagctccgggttgggctgagatggctgtgccccaactcccattcacccaccatggacccaataataaacctggccccacccc

SEQ ID NO: 2 - protein, 185 aa, Homo sapiens
MRLLTLLGLLCGSVATPLGPKWPEPVFGRLASPGFPGEYANDQERRWTLTAPPGYRLRLYFTHFDLELSHLCEYDFVKLSSGAKVLATLCGQESTDTERAPGKDTFYSLGSSLDITFRSDYSNEKPFTGFEAFYAAEDIDECQVAPGEAPTCDHHCHNHLGGFYCSCRAGYVLHRNKRTCSEQSL

SEQ ID NO: 3 - protein, 170 aa, Homo sapiens
TPLGPKWPEPVFGRLASPGFPGEYANDQERRWTLTAPPGYRLRLYFTHFDLELSHLCEYDFVKLSSGAKVLATLCGQESTDTERAPGKDTFYSLGSSLDITFRSDYSNEKPFTGFEAFYAAEDIDECQVAPGEAPTCDHHCHNHLGGFYCSCRAGYVLHRNKRTCSEQSL

SEQ ID NO: 4 - DNA, 2460 bp, Homo sapiens
  CDS (22)..(2082)
ggccagctggacgggcacaccatgaggctgctgaccctcctgggccttctgtgtggctcggtggccacccccttgggcccgaagtggcctgaacctgtgttcgggcgcctggcatcccccggctttccaggggagtatgccaatgaccaggagcggcgctggaccctgactgcaccccccggctaccgcctgcgcctctacttcacccacttcgacctggagctctcccacctctgcgagtacgacttcgtcaagctgagctcgggggccaaggtgctggccacgctgtgcgggcaggagagcacagacacggagcgggcccctggcaaggacactttctactcgctgggctccagcctggacattaccttccgctccgactactccaacgagaagccgttcacggggttcgaggccttctatgcagccgaggacattgacgagtgccaggtggccccgggagaggcgcccacctgcgaccaccactgccacaaccacctgggcggtttctactgctcctgccgcgcaggctacgtcctgcaccgtaacaagcgcacctgctcagccctgtgctccggccaggtcttcacccagaggtctggggagctcagcagccctgaatacccacggccgtatcccaaactctccagttgcacttacagcatcagcctggaggaggggttcagtgtcattctggactttgtggagtccttcgatgtggagacacaccctgaaaccctgtgtccctacgactttctcaagattcaaacagacagagaagaacatggcccattctgtgggaagacattgccccacaggattgaaacaaaaagcaacacggtgaccatcacctttgtcacagatgaatcaggagaccacacaggctggaagatccactacacgagcacagcgcagccttgcccttatccgatggcgccacctaatggccacgtttcacctgtgcaagccaaatacatcctgaaagacagcttctccatcttttgcgagactggctatgagcttctgcaaggtcacttgcccctgaaatcctttactgcagtttgtcagaaagatggatcttgggaccggccaatgcccgcgtgcagcattgttgactgtggccctcctgatgatctacccagtggccgagtggagtacatcacaggtcctggagtgaccacctacaaagctgtgattcagtacagctgtgaagagaccttctacacaatgaaagtgaatgatggtaaatatgtgtgtgaggctgatggattctggacgagctccaaaggagaaaaatcactcccagtctgtgagcctgtttgtggactatcagcccgcacaacaggagggcgtatatatggagggcaaaaggcaaaacctggtgattttccttggcaagtcctgatattaggtggaaccacagcagcaggtgcacttttatatgacaactgggtcctaacagctgctcatgccgtctatgagcaaaaacatgatgcatccgccctggacattcgaatgggcaccctgaaaagactatcacctcattatacacaagcctggtctgaagctgtttttatacatgaaggttatactcatgatgctggctttgacaatgacatagcactgattaaattgaataacaaagttgtaatcaatagcaacatcacgcctatttgtctgccaagaaaagaagctgaatcctttatgaggacagatgacattggaactgcatctggatggggattaacccaaaggggttttcttgctagaaatctaatgtatgtcgacataccgattgttgaccatcaaaaatgtactgctgcatatgaaaagccaccctatccaaggggaagtgtaactgctaacatgctttgtgctggcttagaaagtgggggcaaggacagctgcagaggtgacagcggaggggcactggtgtttctagatagtgaaacagagaggtggtttgtgggaggaatagtgtcctggggttccatgaattgtggggaagcaggtcagtatggagtctacacaaaagttattaactatattccctggatcgagaacataattagtgatttttaacttgcgtgtctgcagtcaaggattcttcatttttagaaatgcctgtgaagaccttggcagcgacgtggctcgagaagcattcatcattactgtggacatggcagttgttgctccacccaaaaaaacagactccaggtgaggctgctgtcatttctccacttgccagtttaattccagccttacccattgactcaaggggacataaaccacgagagtgacagtcatctttgcccacccagtgtaatgtcactgctcaaattacatttcattaccttaaaaagccagtctcttttcatactggctgttggcatttctgtaaactgcctgtccatgctctttgtttttaaacttgttcttattgaaaaaaaaaaaaaaaaa

SEQ ID NO: 5 - protein, 686 aa, Homo sapiens
MRLLTLLGLLCGSVATPLGPKWPEPVFGRLASPGFPGEYANDQERRWTLTAPPGYRLRLYFTHFDLELSHLCEYDFVKLSSGAKVLATLCGQESTDTERAPGKDTFYSLGSSLDITFRSDYSNEKPFTGFEAFYAAEDIDECQVAPGEAPTCDHHCHNHLGGFYCSCRAGYVLHRNKRTCSALCSGQVFTQRSGELSSPEYPRPYPKLSSCTYSISLEEGFSVILDFVESFDVETHPETLCPYDFLKIQTDREEHGPFCGKTLPHRIETKSNTVTITFVTDESGDHTGWKIHYTSTAQPCPYPMAPPNGHVSPVQAKYILKDSFSIFCETGYELLQGHLPLKSFTAVCQKDGSWDRPMPACSIVDCGPPDDLPSGRVEYITGPGVTTYKAVIQYSCEETFYTMKVNDGKYVCEADGFWTSSKGEKSLPVCEPVCGLSARTTGGRIYGGQKAKPGDFPWQVLILGGTTAAGALLYDNWVLTAAHAVYEQKHDASALDIRMGTLKRLSPHYTQAWSEAVFIHEGYTHDAGFDNDIALIKLNNKVVINSNITPICLPRKEAESFMRTDDIGTASGWGLTQRGFLARNLMYVDIPIVDHQKCTAAYEKPPYPRGSVTANMLCAGLESGGKDSCRGDSGGALVFLDSETERWFVGGIVSWGSMNCGEAGQYGVYTKVINYIPWIENIISDF

SEQ ID NO: 6 - protein, 671 aa, Homo sapiens
TPLGPKWPEPVFGRLASPGFPGEYANDQERRWTLTAPPGYRLRLYFTHFDLELSHLCEYDFVKLSSGAKVLATLCGQESTDTERAPGKDTFYSLGSSLDITFRSDYSNEKPFTGFEAFYAAEDIDECQVAPGEAPTCDHHCHNHLGGFYCSCRAGYVLHRNKRTCSALCSGQVFTQRSGELSSPEYPRPYPKLSSCTYSISLEEGFSVILDFVESFDVETHPETLCPYDFLKIQTDREEHGPFCGKTLPHRIETKSNTVTITFVTDESGDHTGWKIHYTSTAQPCPYPMAPPNGHVSPVQAKYILKDSFSIFCETGYELLQGHLPLKSFTAVCQKDGSWDRPMPACSIVDCGPPDDLPSGRVEYITGPGVTTYKAVIQYSCEETFYTMKVNDGKYVCEADGFWTSSKGEKSLPVCEPVCGLSARTTGGRIYGGQKAKPGDFPWQVLILGGTTAAGALLYDNWVLTAAHAVYEQKHDASALDIRMGTLKRLSPHYTQAWSEAVFIHEGYTHDAGFDNDIALIKLNNKVVINSNITPICLPRKEAESFMRTDDIGTASGWGLTQRGFLARNLMYVDIPIVDHQKCTAAYEKPPYPRGSVTANMLCAGLESGGKDSCRGDSGGALVFLDSETERWFVGGIVSWGSMNCGEAGQYGVYTKVINYIPWIENIISDF

SEQ ID NO: 7 - DNA, 4900 bp, Homo sapiens
cctgtcctgcctgcctggaactctgagcaggctggagtcatggagtcgattcccagaatcccagagtcagggaggctgggggcaggggcaggtcactggacaaacagatcaaaggtgagaccagcgtaggactgcagaccaggccaggccagctggacgggcacaccatgaggtaggtgggcgccacagcctccctgcagggtgtggggtgggagcacaggcctgggcctcaccgcccctgccctgcccataggctgctgaccctcctgggccttctgtgtggctcggtggccacccccttaggcccgaagtggcctgaacctgtgttcgggcgcctggcatcccccggctttccaggggagtatgccaatgaccaggagcggcgctggaccctgactgcaccccccggctaccgcctgcgcctctacttcacccacttcgacctggagctctcccacctctgcgagtacgacttcgtcaaggtgccgtcagacgggagggctggggtttctcagggtcggggggtccccaaggagtagccagggttcagggacacctgggagcaggggccaggcttggccaggagggagatcaggcctgggtcttgccttcactccctgtgacacctgaccccacagctgagctcgggggccaaggtgctggccacgctgtgcgggcaggagagcacagacacggagcgggcccctggcaaggacactttctactcgctgggctccagcctggacattaccttccgctccgactactccaacgagaagccgttcacggggttcgaggccttctatgcagccgagggtgagccaagaggggtcctgcaacatctcagtctgcgcagctggctgtgggggtaactctgtcttaggccaggcagccctgccttcagtttccccacctttcccagggcaggggagaggcctctggcctgacatcatccacaatgcaaagaccaaaacagccgtgacctccattcacatgggctgagtgccaactctgagccagggatctgaggacagcatcgcctcaagtgacgcagggactggccgggcgcggcagctcacgcctgtaattccagcactttgggaggccgaggctggcttgataatttgagggtcaggagttcaaggccagccagggcaacacggtgaaactctatctccactaaaactacaaaaattagctgggcgtggtggtgcgcacctggaatcccagctactagggaggctgaggcaggagaattgcttgaacctgcgaggtggaggctgcagtgaacagagattgcaccactacactccacctgggcgacagactagactccgtctcaaaaaacaaaaaacaaaaaccacgcagggccgagggcccatttacaagctgacaaagtgggccctgccagcgggagcgctgcaggatgtttgattttcagatcccagtccctgcagagaccaactgtgtgacctctggcaagtggctcaatttctctgctccttagaagctgctgcaagggttcagcgctgtagccccgccccctgggtttgattgactcccctcattagctgggtgacctcggccggacactgaaactcccactggtttaacagaggtgatgtttgcatctttctcccagcgctgctgggagcttgcagcgaccctaggcctgtaaggtgattggcccggcaccagtcccgcaccctagacaggacctaggcctcctctgaggtccactctgaggtcatggatctcctgggaggagtccaggctggatcccgcctctttccctcctgacggcctgcctggccctgcctctcccccagacattgacgagtgccaggtggccccgggagaggcgcccacctgcgaccaccactgccacaaccacctgggcggtttctactgctcctgccgcgcaggctacgtcctgcaccgtaacaagcgcacctgctcaggtgagggaggctgcctgggccccaacgcaccctctcctgggatacccggggctcctcagggccattgctgctctgcccaggggtgcggagggcctgggcctggacactgggtgcttctaggccctgctgcctccagctccccttctcagccctgcttcccctctcagcagccaggctcatcagtgccaccctgccctagcactgagactaattctaacatcccactgtgtacctggttccacctgggctctgggaacccctcatgtagccacgggagagtcggggtatctaccctcgttccttggactgggttcctgttccctgcactgggggacgggccagtgctctggggcgtgggcagccccaccctgtggcgctgaccctgctcccccgactcggtttctcctctcggggtctctccttgcctctctgatctctcttccagagcagagcctctagcctcccctggagctccggctgcccagcaggtcagaagccagagccaggctgctggcctcagctccgggttgggctgagatgctgtgccccaactcccattcacccaccatggacccaataataaacctggccccaccccacctgctgccgcgtgtctctggggtgggagggtcgggaggcggtggggcgcgctcctctctgcctaccctcctcacagcctcatgaaccccaggtctgtgggagcctcctccatggggccacacggtccttggcctcaccccctgttttgaagatggggcactgaggccggagaggggtaaggcctcgctcgagtccaggtccccagaggctgagcccagagtaatcttgaaccacccccattcagggtctggcctggaggagcctgacccacagaggagacaccctgggagatattcattgaggggtaatctggtcccccgcaaatccaggggtgattcccactgccccataggcacagccacgtggaagaaggcaggcaatgttggggctcctcacttcctagaggcctcacaactcaaatgccccccactgcagctgggggtggggtggtggtatgggatggggaccaagccttccttgaaggatagagcccagcccaacaccccgccccgtggcagcagcatcacgtgttccagcgaggaaggagagcaccagactcagtcatgatcactgttgccttgaacttccaagaacagccccagggcaagggtcaaaacaggggaaagggggtgatgagagatccttcttccggatgttcctccaggaaccagggggctggctggtcttggctgggttcgggtaggagacccatgatgaataaacttgggaatcactggggtggctgtaagggaatttaggggagctccgaaggggcccttaggctcgaggagatgctcctctcttttcccgaattcccagggacccaggagagtgtcccttcttcctcttcctgtgtgtccatccacccccgccccccgccctggcagagctggtggaactcagtgctctagcccctaccctggggttgcgactctggctcaggacaccaccacgctccctgggggtgtgagtgagggcctgtgcgctccatcccgagtgctgcctgtttcagctaaagcctcaaagcaagagaaaccccctctctaagcggcccctcagccatcgggtgggtcgtttggtttctgggtaggcctcaggggctggccacctgcagggcccagcccaacccagggatgcagatgtcccagccacatccctgtcccagtttcctgctccccaaggcatccaccctgctgttggtgcgagggctgatagagggcacgccaagtcactcccctgcccttccctccttccagccctgtgctccggccaggtcttcacccagaggtctggggagctcagcagccctgaatacccacggccgtatcccaaactctccagttgcacttacagcatcagcctggaggaggggttcagtgtcattctggactttgtggagtccttcgatgtggagacacaccctgaaaccctgtgtccctacgactttctcaaggtctggctcctgggcccctcatcttgtcccagatcctcccccttcagcccagctgcaccccctacttcctgcagcatggcccccaccacgttcccgtcaccctcggtgaccccacctcttcaggtgctctatggaggtcaaggctggggcttcgagtacaagtgtgggaggcagagtggggaggggcaccccaatccatggcctgggttggcctcattggctgtccctgaaatgctgaggaggtgggttacttccctccgcccaggccagacccaggcagctgctccccagctttcatgagcttctttctcagattcaaacagacagagaagaacatggcccattctgtgggaagacattgccccacaggattgaaacaaaaagcaacacggtgaccatcacctttgtcacagatgaatcaggagaccacacaggctggaagatccactacacgagcacagtgagcaagtgggctcagatccttggtggaagcgcagagctgcctctctctggagtgcaaggagctgtagagtgtagggctcttctgggcaggactaggaagggacaccaggtttagtggtgctgaggtctgaggcagcagcttctaaggggaagcacccgtgccctcctcagcagcacccagcatcttcaccactcattcttcaaccacccattcacccatcactcatcttttacccacccaccctttgccactcatccttctgtccctcatccttccaaccattcatcaatcacccacccatccatcctttgccacacaaccatccacccattcttctacctacccatcctatccatccatccttctatcagcatccttctaccacccatccttcgttcggtcatccatcatcatccatccatc

SEQ ID NO: 8 - protein, 136 aa, Homo sapiens
MRLLTLLGLLCGSVATPLGPKWPEPVFGRLASPGFPGEYANDQERRWTLTAPPGYRLRLYFTHFDLELSHLCEYDFVKLSSGAKVLATLCGQESTDTERAPGKDTFYSLGSSLDITFRSDYSNEKPFTGFEAFYAA

SEQ ID NO: 9 - protein, 181 aa, Homo sapiens
MRLLTLLGLLCGSVATPLGPKWPEPVFGRLASPGFPGEYANDQERRWTLTAPPGYRLRLYFTHFDLELSHLCEYDFVKLSSGAKVLATLCGQESTDTERAPGKDTFYSLGSSLDITFRSDYSNEKPFTGFEAFYAAEDIDECQVAPGEAPTCDHHCHNHLGGFYCSCRAGYVLHRNKRTCS

SEQ ID NO: 10 - protein, 293 aa, Homo sapiens
MRLLTLLGLLCGSVATPLGPKWPEPVFGRLASPGFPGEYANDQERRWTLTAPPGYRLRLYFTHFDLELSHLCEYDFVKLSSGAKVLATLCGQESTDTERAPGKDTFYSLGSSLDITFRSDYSNEKPFTGFEAFYAAEDIDECQVAPGEAPTCDHHCHNHLGGFYCSCRAGYVLHRNKRTCSALCSGQVFTQRSGELSSPEYPRPYPKLSSCTYSISLEEGFSVILDFVESFDVETHPETLCPYDFLKIQTDREEHGPFCGKTLPHRIETKSNTVTITFVTDESGDHTGWKIHY

SEQ ID NO: 11 - protein, 41 aa, Homo sapiens
EDIDECQVAPGEAPTCDHHCHNHLGGFYCSCRAGYVLHRNK

SEQ ID NO: 12 - protein, 242 aa, Homo sapiens
IYGGQKAKPGDFPWQVLILGGTTAAGALLYDNWVLTAAHAVYEQKHDASALDIRMGTLKRLSPHYTQAWSEAVFIHEGYTHDAGFDNDIALIKLNNKVVINSNITPICLPRKEAESFMRTDDIGTASGWGLTQRGFLARNLMYVDIPIVDHQKCTAAYEKPPYPRGSVTANMLCAGLESGGKDSCRGDSGGALVFLDSETERWFVGGIVSWGSMNCGEAGQYGVYTKVINYIPWIENIISDF

SEQ ID NO: 13 - protein, 16 aa, Artificial Sequence
  Synthetic
GKDSCRGDAGGALVFL

SEQ ID NO: 14 - protein, 15 aa, Artificial Sequence
  Synthetic
TPLGPKWPEPVFGRL

SEQ ID NO: 15 - protein, 43 aa, Artificial Sequence
  Synthetic
TAPPGYRLRLYFTHFDLELSHLCEYDFVKLSSGAKVLATLCGQ

SEQ ID NO: 16 - protein, 8 aa, Artificial Sequence
  Synthetic
TFRSDYSN

SEQ ID NO: 17 - protein, 25 aa, Artificial Sequence
  Synthetic
FYSLGSSLDITFRSDYSNEKPFTGF

SEQ ID NO: 18 - protein, 9 aa, Artificial Sequence
  Synthetic
IDECQVAPG

SEQ ID NO: 19 - protein, 25 aa, Artificial Sequence
  Synthetic
ANMLCAGLESGGKDSCRGDSGGALV

SEQ ID NO: 20 - DNA, 960 bp, Homo sapiens
  CDS (51)..(797)
attaactgagattaaccttccctgagttttctcacaccaaggtgaggaccatgtccctgtttccatcactccctctccttctcctgagtatggtggcagcgtcttactcagaaactgtgacctgtgaggatgcccaaaagacctgccctgcagtgattgcctgtagctctccaggcatcaacggcttcccaggcaaagatgggcgtgatggcaccaagggagaaaagggggaaccaggccaagggctcagaggcttacagggcccccctggaaagttggggcctccaggaaatccagggccttctgggtcaccaggaccaaagggccaaaaaggagaccctggaaaaagtccggatggtgatagtagcctggctgcctcagaaagaaaagctctgcaaacagaaatggcacgtatcaaaaagtggctcaccttctctctgggcaaacaagttgggaacaagttcttcctgaccaatggtgaaataatgacctttgaaaaagtgaaggccttgtgtgtcaagttccaggcctctgtggccacccccaggaatgctgcagagaatggagccattcagaatctcatcaaggaggaagccttcctgggcatcactgatgagaagacagaagggcagtttgtggatctgacaggaaatagactgacctacacaaactggaacgagggtgaacccaacaatgctggttctgatgaagattgtgtattgctactgaaaaatggccagtggaatgacgtcccctgctccacctcccatctggccgtctgtgagttccctatctgaagggtcatatcactcaggccctccttgtctttttactgcaacccacaggcccacagtatgcttgaaaagataaattatatcaatttcctcatatccagtattgttccttttgtgggcaatcactaaaaatgatcactaacagcaccaacaaagcaataatagt

SEQ ID NO: 21 - protein, 248 aa, Homo sapiens
MSLFPSLPLLLLSMVAASYSETVTCEDAQKTCPAVIACSSPGINGFPGKDGRDGTKGEKGEPGQGLRGLQGPPGKLGPPGNPGPSGSPGPKGQKGDPGKSPDGDSSLAASERKALQTEMARIKKWLTFSLGKQVGNKFFLTNGEIMTFEKVKALCVKFQASVATPRNAAENGAIQNLIKEEAFLGITDEKTEGQFVDLTGNRLTYTNWNEGEPNNAGSDEDCVLLLKNGQWNDVPCSTSHLAVCEFPI

SEQ ID NO: 22 - protein, 6 aa, Artificial Sequence
  Synthetic
  MISC_FEATURE (1)..(1): Wherein X at position 1 represents hydroxyproline
  MISC_FEATURE (4)..(4): Wherein X at position 4 represents hydrophobic residue
XGKXGP

SEQ ID NO: 23 - protein, 5 aa, Artificial Sequence
  Synthetic
  MISC_FEATURE (1)..(1): Wherein X represents hydroxyproline
XGKLG

SEQ ID NO: 24 - protein, 16 aa, Artificial Sequence
  Synthetic
  MISC_FEATURE (9)..(15): Wherein X at positions 9 and 15 represents hydroxyproline
GLRGLQGPXGKLGPXG

SEQ ID NO: 25 - protein, 27 aa, Artificial Sequence
  Synthetic
  MISC_FEATURE (3)..(27): Wherein X at positions 3, 6, 15, 21, 24, 27 represents hydroxyproline
GPXGPXGLRGLQGPXGKLGPXGPXGPX

SEQ ID NO: 26 - protein, 53 aa, Artificial Sequence
  Synthetic
  misc_feature (26)..(26): Xaa can be any naturally occurring amino acid
  misc_feature (32)..(32): Xaa can be any naturally occurring amino acid
  misc_feature (35)..(35): Xaa can be any naturally occurring amino acid
  misc_feature (41)..(41): Xaa can be any naturally occurring amino acid
  misc_feature (50)..(50): Xaa can be any naturally occurring amino acid
GKDGRDGTKGEKGEPGQGLRGLQGPXGKLGPXGNXGPSGSXGPKGQKGDXGKS

SEQ ID NO: 27 - protein, 33 aa, Artificial Sequence
  Synthetic
  MISC_FEATURE (3)..(33): Wherein X at positions 3, 6, 12, 18, 21, 30, 33 represents hydroxyproline
GAXGSXGEKGAXGPQGPXGPXGKMGPKGEXGDX

SEQ ID NO: 28 - protein, 45 aa, Artificial Sequence
  Synthetic
  MISC_FEATURE (3)..(45): Wherein X at positions 3, 6, 9, 27, 30, 36, 42, 45 represents hydroxyproline
GCXGLXGAXGDKGEAGTNGKRGERGPXGPXGKAGPXGPNGAXGEX

SEQ ID NO: 29 - protein, 24 aa, Artificial Sequence
  Synthetic
LQRALEILPNRVTIKANRPFLVFI

SEQ ID NO: 30 - DNA, 559 bp, Homo sapiens
atgaggctgctgaccctcctgggccttctgtgtggctcggtggccacccccttgggcccgaagtggcctgaacctgtgttcgggcgcctggcatcccccggctttccaggggagtatgccaatgaccaggagcggcgctggaccctgactgcaccccccggctaccgcctgcgcctctacttcacccacttcgacctggagctctcccacctctgcgagtacgacttcgtcaagctgagctcgggggccaaggtgctggccacgctgtgcgggcaggagagcacagacacggagcgggcccctggcaaggacactttctactcgctgggctccagcctggacattaccttccgctccgactactccaacgagaagccgttcacggggttcgaggccttctatgcagccgaggacattgacgagtgccaggtggccccgggagaggcgcccacctgcgaccaccactgccacaaccacctgggcggtttctactgctcctgccgcgcaggctacgtcctgcaccgtaacaagcgcacctgctcagccctgtgctccggcc

SEQ ID NO: 31 - DNA, 34 bp, Artificial Sequence
  Synthetic
cgggcacaccatgaggctgctgaccctcctgggc

SEQ ID NO: 32 - DNA, 33 bp, Artificial Sequence
  Synthetic
gacattaccttccgctccgactccaacgagaag

SEQ ID NO: 33 - DNA, 33 bp, Artificial Sequence
  Synthetic
agcagccctgaatacccacggccgtatcccaaa

SEQ ID NO: 34 - DNA, 26 bp, Artificial Sequence
  Synthetic
cgggatccatgaggctgctgaccctc

SEQ ID NO: 35 - DNA, 19 bp, Artificial Sequence
  Synthetic
ggaattcctaggctgcata

SEQ ID NO: 36 - DNA, 19 bp, Artificial Sequence
  Synthetic
ggaattcctacagggcgct

SEQ ID NO: 37 - DNA, 19 bp, Artificial Sequence
  Synthetic
ggaattcctagtagtggat

SEQ ID NO: 38 - DNA, 25 bp, Artificial Sequence
  Synthetic
tgcggccgctgtaggtgctgtcttt

SEQ ID NO: 39 - DNA, 23 bp, Artificial Sequence
  Synthetic
ggaattcactcgttattctcgga

SEQ ID NO: 40 - DNA, 17 bp, Artificial Sequence
  Synthetic
tccgagaataacgagtg

SEQ ID NO: 41 - DNA, 29 bp, Artificial Sequence
  Synthetic
cattgaaagctttggggtagaagttgttc

SEQ ID NO: 42 - DNA, 27 bp, Artificial Sequence
  Synthetic
cgcggccgcagctgctcagagtgtaga

SEQ ID NO: 43 - DNA, 28 bp, Artificial Sequence
  Synthetic
cggtaagcttcactggctcagggaaata

SEQ ID NO: 44 - DNA, 37 bp, Artificial Sequence
  Synthetic
aagaagcttgccgccaccatggattggctgtggaact

SEQ ID NO: 45 - DNA, 31 bp, Artificial Sequence
  Synthetic
cgggatcctcaaactttcttgtccaccttgg

SEQ ID NO: 46 - DNA, 36 bp, Artificial Sequence
  Synthetic
aagaaagcttgccgccaccatgttctcactagctct

SEQ ID NO: 47 - DNA, 26 bp, Artificial Sequence
  Synthetic
cgggatccttctccctctaacactct

SEQ ID NO: 48 - protein, 9 aa, Artificial Sequence
  Synthetic
EPKSCDKTH

SEQ ID NO: 49 - DNA, 4960 bp, Homo Sapiens
ccggacgtggtggcgcatgcctgtaatcccagctactcgggaggctgaggcaggagaattgctcgaaccccggaggcagaggtttggtggctcacacctgtaatcccagcactttgcgaggctgaggcaggtgcatcgctttggctcaggagttcaagaccagcctgggcaacacagggagacccccatctctacaaaaaacaaaaacaaatataaaggggataaaaaaaaaaaaaagacaagacatgaatccatgaggacagagtgtggaagaggaagcagcagcctcaaagttctggaagctggaagaacagataaacaggtgtgaaataactgcctggaaagcaacttctttttttttttttttttttttgaggtggagtctcactctgtcgtccaggctggagtgcagtggtgcgatctcggatcactgcaacctccgcctcccaggctcaagcaattctcctgcctcagcctcccgagtagctgggattataagtgcgcgctgccacacctggatgatttttgtatttttagtagagatgggatttcaccatgttggtcaggctggtctcaaactcccaacctcgtgatccacccaccttggcctcccaaagtgctgggattacaggtataagccaccgagcccagccaaaagcgacttctaagcctgcaagggaatcgggaattggtggcaccaggtccttctgacagggtttaagaaattagccagcctgaggctgggcacggtggctcacacctgtaatcccagcactttgggaggctaaggcaggtggatcacctgagggcaggagttcaagaccagcctgaccaacatggagaaaccccatccctaccaaaaataaaaaattagccaggtgtggtggtgctcgcctgtaatcccagctacttgggaggctgaggtgggaggattgcttgaacacaggaagtagaggctgcagtgagctatgattgcagcactgcactgaagccggggcaacagaacaagatccaaaaaaaagggaggggtgaggggcagagccaggatttgtttccaggctgttgttacctaggtccgactcctggctcccagagcagcctgtcctgcctgcctggaactctgagcaggctggagtcatggagtcgattcccagaatcccagagtcagggaggctgggggcaggggcaggtcactggacaaacagatcaaaggtgagaccagcgtagggctgcagaccaggccaggccagctggacgggcacaccatgaggtaggtgggcgcccacagcctccctgcagggtgtggggtgggagcacaggcctgggccctcaccgcccctgccctgcccataggctgctgaccctcctgggccttctgtgtggctcggtggccacccccttgggcccgaagtggcctgaacctgtgttcgggcgcctggcatcccccggctttccaggggagtatgccaatgaccaggagcggcgctggaccctgactgcaccccccggctaccgcctgcgcctctacttcacccacttcgacctggagctctcccacctctgcgagtacgacttcgtcaaggtgccgtcaggacgggagggctggggtttctcagggtcggggggtccccaaggagtagccagggttcagggacacctgggagcaggggccaggcttggccaggagggagatcaggcctgggtcttgccttcactccctgtgacacctgaccccacagctgagctcgggggccaaggtgctggccacgctgtgcgggcaggagagcacagacacggagcgggcccctggcaaggacactttctactcgctgggctccagcctggacattaccttccgctccgactactccaacgagaagccgttcacggggttcgaggccttctatgcagccgagggtgagccaagaggggtcctgcaacatctcagtctgcgcagctggctgtgggggtaactctgtcttaggccaggcagccctgccttcagtttccccacctttcccagggcaggggagaggcctctggcctgacatcatccacaatgcaaagaccaaaacagccgtgacctccattcacatgggctgagtgccaactctgagccagggatctgaggacagcatcgcctcaagtgacgcagggactggccgggcgcagcagctcacgcctgtaattccagcactttgggaggccgaggctggctgatcatttgaggtcaggagttcaaggccagccagggcaacacggtgaaactctatctccactaaaactacaaaaattagctgggcgtggtggtgcgcacctggaatcccagctactagggaggctgaggcaggagaattgcttgaacctgcgaggtggaggctgcagtgaacagagattgcaccactacactccagcctgggcgacagagctagactccgtctcaaaaaacaaaaaacaaaaacgacgcaggggccgagggccccatttacagctgacaaagtggggccctgccagcgggagcgctgccaggatgtttgatttcagatcccagtccctgcagagaccaactgtgtgacctctggcaagtggctcaatttctctgctccttaggaagctgctgcaagggttcagcgctgtagccccgccccctgggtttgattgactcccctcattagctgggtgacctcgggccggacactgaaactcccactggtttaacagaggtgatgtttgcatctttctcccagcgctgctgggagcttgcagcgaccctaggcctgtaaggtgattggcccggcaccagtcccgcaccctagacaggacgaggcctcctctgaggtccactctgaggtcatggatctcctgggaggagtccaggctggatcccgcctctttccctcctgacggcctgcctggccctgcctctcccccagacattgacgagtgccaggtggccccgggagaggcgcccacctgcgaccaccactgccacaaccacctgggcggtttctactgctcctgccgcgcaggctacgtcctgcaccgtaacaagcgcacctgctcagccctgtgctccggccaggtcttcacccagaggtctggggagctcagcagccctgaatacccacggccgtatcccaaactctccagttgcacttacagcatcagcctggaggaggggttcagtgtcattctggactttgtggagtccttcgatgtggagacacaccctgaaaccctgtgtccctacgactttctcaagattcaaacagacagagaagaacatggcccattctgtgggaagacattgccccacaggattgaaacaaaaagcaacacggtgaccatcacctttgtcacagatgaatcaggagaccacacaggctggaagatccactacacgagcacagcgcacgcttgcccttatccgatggcgccacctaatggccacgtttcacctgtgcaagccaaatacatcctgaaagacagcttctccatcttttgcgagactggctatgagcttctgcaaggtcacttgcccctgaaatcctttactgcagtttgtcagaaagatggatcttgggaccggccaatgcccgcgtgcagcattgttgactgtggccctcctgatgatctacccagtggccgagtggagtacatcacaggtcctggagtgaccacctacaaagctgtgattcagtacagctgtgaagagaccttctacacaatgaaagtgaatgatggtaaatatgtgtgtgaggctgatggattctggacgagctccaaaggagaaaaatcactcccagtctgtgagcctgtttgtggactatcagcccgcacaacaggagggcgtatatatggagggcaaaaggcaaaacctggtgattttccttggcaagtcctgatattaggtggaaccacagcagcaggtgcacttttatatgacaactgggtcctaacagctgctcatgccgtctatgagcaaaaacatgatgcatccgccctggacattcgaatgggcaccctgaaaagactatcacctcattatacacaagcctggtctgaagctgtttttatacatgaaggttatactcatgatgctggctttgacaatgacatagcactgattaaattgaataacaaagttgtaatcaatagcaacatcacgcctatttgtctgccaagaaaagaagctgaatcctttatgaggacagatgacattggaactgcatctggatggggattaacccaaaggggttttcttgctagaaatctaatgtatgtcgacataccgattgttgaccatcaaaaatgtactgctgcatatgaaaagccaccctatccaaggggaagtgtaactgctaacatgctttgtgctggcttagaaagtgggggcaaggacagctgcagaggtgacagcggaggggcactggtgtttctagatagtgaaacagagaggtggtttgtgggaggaatagtgtcctggggttccatgaattgtggggaagcaggtcagtatggagtctacacaaaagttattaactatattccctggatcgagaacataattagtgatttttaacttgcgtgtctgcagtcaaggattcttcatttttagaaatgcctgtgaagaccttggcagcgacgtggctcgagaagcattcatcattactgtggacatggcagttgttgctccacccaaaaaaacagactccaggtgaggctgctgtcatttctccacttgccagtttaattccagccttacccattgactcaaggggacataaaccacgagagtgacagtcatctttgcccacccagtgtaatgtcactgctcaaattacatttcattaccttaaaaagccagtctcttttcatactggctgttggcatttctgtaaactgcctgtccatgctctttgtttttaaacttgttcttattgaaaaaaaaaaaaaaaaa

SEQ ID NO: 50 - DNA, 2090 bp, Murine
  CDS (33)..(2090)
ggcgctggactgcagagctatggtggcacaccatgaggctactcatcttcctgggtctgctgtggagtttggtggccacacttctgggttcaaagtggcctgaacctgtattcgggcgcctggtgtcccctggcttcccagagaagtatgctgaccatcaagatcgatcctggacactgactgcaccccctggctaccgcctgcgcctctacttcacccactttgacctggaactctcttaccgctgcgagtatgactttgtcaagttgagctcagggaccaaggtgctggccacactgtgtgggcaggagagtacagacactgagcaggcacctggcaatgacaccttctactcactgggtcccagcctaaaggtcaccttccactccgactactccaatgagaagccgttcacagggtttgaggccttctatgcagcggaggatgtggatgaatgcagagtgtctctgggagactcagtcccttgtgaccattattgccacaactacttgggcggctactattgctcctgcagagcgggctacattctccaccagaacaagcacacgtgctcagccctttgttcaggccaggtgttcacaggaagatctgggtatctcagtagccctgagtacccgcagccataccccaagctctccagctgcacctacagcatccgcctggaggacggcttcagtgtcatcctggacttcgtggagtccttcgatgtggagacgcaccctgaagcccagtgcccctatgactccctcaagattcaaacagacaagggggaacacggcccattttgtgggaagacgctgcctcccaggattgaaactgacagccacaaggtgaccatcacctttgccactgacgagtcggggaaccacacaggctggaagatacactacacaagcacagcacggccctgccctgatccaacggcgccacctaatggcagcatttcacctgtgcaagccacgtatgtcctgaaggacaggttttctgtcttctgcaagacaggcttcgagcttctgcaaggttctgtccccctgaaatcattcactgctgtctgtcagaaagatggatcttgggaccggccgatgccagagtgcagcattattgattgtggccctcccgatgacctacccaatggccatgtggactatatcacaggccctcaagtgactacctacaaagctgtgattcagtacagctgtgaagagactttctacacaatgagcagcaatggtaaatatgtgtgtgaggctgatggattctggacgagctccaaaggagaaaaactccccccggtttgtgagcctgtttgtgggctgtccacacacactataggaggacgcatagttggagggcagcctgcaaagcctggtgactttccttggcaagtcttgttgctgggtcaaactacagcagcagcaggtgcacttatacatgacaattgggtcctaacagccgctcatgctgtatatgagaaaagaatggcagcgtcctccctgaacatccgaatgggcatcctcaaaaggctctcacctcattacactcaagcctggcccgaggaaatctttatacatgaaggctacactcacggtgctggttttgacaatgatatagcattgattaaactcaagaacaaagtcacaatcaacggaagcatcatgcctgtttgcctaccgcgaaaagaagctgcatccttaatgagaacagacttcactggaactgtggctggctgggggttaacccagaaggggcttcttgctagaaacctaatgtttgtggacataccaattgctgaccaccaaaaatgtaccaccgtgtatgaaaagctctatccaggagtaagagtaagcgctaacatgctctgtgctggcttagagactggtggcaaggacagctgcagaggtgacagtgggggggcattagtgtttctagataatgagacacagcgatggtttgtgggaggaatagtttcctggggttccattaattgtggggcggcaggccagtatggggtctacacaaaagtcatcaactatattccctggaatgagaacataataagtaatttctaa

SEQ ID NO: 51 - protein, 685 aa, Murine
MRLLIFLGLLWSLVATLLGSKWPEPVFGRLVSPGFPEKYADHQDRSWTLTAPPGYRLRLYFTHFDLELSYRCEYDFVKLSSGTKVLATLCGQESTDTEQAPGNDTFYSLGPSLKVTFHSDYSNEKPFTGFEAFYAAEDVDECRVSLGDSVPCDHYCHNYLGGYYCSCRAGYILHQNKHTCSALCSGQVFTGRSGYLSSPEYPQPYPKLSSCTYSIRLEDGFSVILDFVESFDVETHPEAQCPYDSLKIQTDKGEHGPFCGKTLPPRIETDSHKVTITFATDESGNHTGWKIHYTSTARPCPDPTAPPNGSISPVQATYVLKDRFSVFCKTGFELLQGSVPLKSFTAVCQKDGSWDRPMPECSIIDCGPPDDLPNGHVDYITGPQVTTYKAVIQYSCEETFYTMSSNGKYVCEADGFWTSSKGEKLPPVCEPVCGLSTHTIGGRIVGGQPAKPGDFPWQVLLLGQTTAAAGALIHDNWVLTAAHAVYEKRMAASSLNIRMGILKRLSPHYTQAWPEEIFIHEGYTHGAGFDNDIALIKLKNKVTINGSIMPVCLPRKEAASLMRTDFTGTVAGWGLTQKGLLARNLMFVDIPIADHQKCTTVYEKLYPGVRVSANMLCAGLETGGKDSCRGDSGGALVFLDNETQRWFVGGIVSWGSINCGAAGQYGVYTKVINYIPWNENIISNF

SEQ ID NO: 52 - protein, 670 aa, Murine
TLLGSKWPEPVFGRLVSPGFPEKYADHQDRSWTLTAPPGYRLRLYFTHFDLELSYRCEYDFVKLSSGTKVLATLCGQESTDTEQAPGNDTFYSLGPSLKVTFHSDYSNEKPFTGFEAFYAAEDVDECRVSLGDSVPCDHYCHNYLGGYYCSCRAGYILHQNKHTCSALCSGQVFTGRSGYLSSPEYPQPYPKLSSCTYSIRLEDGFSVILDFVESFDVETHPEAQCPYDSLKIQTDKGEHGPFCGKTLPPRIETDSHKVTITFATDESGNHTGWKIHYTSTARPCPDPTAPPNGSISPVQATYVLKDRFSVFCKTGFELLQGSVPLKSFTAVCQKDGSWDRPMPECSIIDCGPPDDLPNGHVDYITGPQVTTYKAVIQYSCEETFYTMSSNGKYVCEADGFWTSSKGEKLPPVCEPVCGLSTHTIGGRIVGGQPAKPGDFPWQVLLLGQTTAAAGALIHDNWVLTAAHAVYEKRMAASSLNIRMGILKRLSPHYTQAWPEEIFIHEGYTHGAGFDNDIALIKLKNKVTINGSIMPVCLPRKEAASLMRTDFTGTVAGWGLTQKGLLARNLMFVDIPIADHQKCTTVYEKLYPGVRVSANMLCAGLETGGKDSCRGDSGGALVFLDNETQRWFVGGIVSWGSINCGAAGQYGVYTKVINYIPWNENIISNF

SEQ ID NO: 53 - DNA, 2091 bp, Rat
  CDS (10)..(2067)
tggcacacaatgaggctactgatcgtcctgggtctgctttggagtttggtggccacacttttgggctccaagtggcctgagcctgtattcgggcgcctggtgtccctggccttcccagagaagtatggcaaccatcaggatcgatcctggacgctgactgcaccccctggcttccgcctgcgcctctacttcacccacttcaacctggaactctcttaccgctgcgagtatgactttgtcaagttgacctcagggaccaaggtgctagccacgctgtgtgggcaggagagtacagatactgagcgggcacctggcaatgacaccttctactcactgggtcccagcctaaaggtcaccttccactccgactactccaatgagaagccattcacaggatttgaggccttctatgcagcggaggatgtggatgaatgcagaacatccctgggagactcagtcccttgtgaccattattgccacaactacctgggcggctactactgctcctgccgagtgggctacattctgcaccagaacaagcatacctgctcagccctttgttcaggccaggtgttcactgggaggtctggctttctcagtagccctgagtacccacagccataccccaaactctccagctgcgcctacaacatccgcctggaggaaggcttcagtatcaccctggacttcgtggagtcctttgatgtggagatgcaccctgaagcccagtgcccctacgactccctcaagattcaaacagacaagagggaatacggcccgttttgtgggaagacgctgccccccaggattgaaactgacagcaacaaggtgaccattacctttaccaccgacgagtcagggaaccacacaggctggaagatacactacacaagcacagcacagccctgccctgatccaacggcgccacctaatggtcacatttcacctgtgcaagccacgtatgtcctgaaggacagcttttctgtcttctgcaagactggcttcgagcttctgcaaggttctgtccccctgaagtcattcactgctgtctgtcagaaagatggatcttgggaccggccgataccagagtgcagcattattgactgtggccctcccgatgacctacccaatggccacgtggactatatcacaggccctgaagtgaccacctacaaagctgtgattcagtacagctgtgaagagactttctacacaatgagcagcaatggtaaatatgtgtgtgaggctgatggattctggacgagctccaaaggagaaaaatccctcccggtttgcaagcctgtctgtggactgtccacacacacttcaggaggccgtataattggaggacagcctgcaaagcctggtgactttccttggcaagtcttgttactgggtgaaactacagcagcaggtgctcttatacatgacgactgggtcctaacagcggctcatgctgtatatgggaaaacagaggcgatgtcctccctggacatccgcatgggcatcctcaaaaggctctccctcatttacactcaagcctggccagaggctgtctttatccatgaaggctacactcacggagctggttttgacaatgatatagcactgattaaactcaagaacaaagtcacaatcaacagaaacatcatgccgatttgtctaccaagaaaagaagctgcatccttaatgaaaacagacttcgttggaactgtggctggctgggggttaacccagaaggggtttcttgctagaaacctaatgtttgtggacataccaattgttgaccaccaaaaatgtgctactgcgtatacaaagcagccctacccaggagcaaaagtgactgttaacatgctctgtgctggcctagaccgcggtggcaaggacagctgcagaggtgacagcggaggggcattagtgtttctagacaatgaaacacagagatggtttgtgggaggaatagtttcctggggttctattaactgtggggggtcagaacagtatggggtctacacgaaagtcacgaactatattccctggattgagaacataataaataatttctaatttgcaaaaaaaaaaaaaaaaaaa

SEQ ID NO: 54 - protein, 685 aa, Rat
MRLLIVLGLLWSLVATLLGSKWPEPVFGRLVSLAFPEKYGNHQDRSWTLTAPPGFRLRLYFTHFNLELSYRCEYDFVKLTSGTKVLATLCGQESTDTERAPGNDTFYSLGPSLKVTFHSDYSNEKPFTGFEAFYAAEDVDECRTSLGDSVPCDHYCHNYLGGYYCSCRVGYILHQNKHTCSALCSGQVFTGRSGFLSSPEYPQPYPKLSSCAYNIRLEEGFSITLDFVESFDVEMHPEAQCPYDSLKIQTDKREYGPFCGKTLPPRIETDSNKVTITFTTDESGNHTGWKIHYTSTAQPCPDPTAPPNGHISPVQATYVLKDSFSVFCKTGFELLQGSVPLKSFTAVCQKDGSWDRPIPECSIIDCGPPDDLPNGHVDYITGPEVTTYKAVIQYSCEETFYTMSSNGKYVCEADGFWTSSKGEKSLPVCKPVCGLSTHTSGGRIIGGQPAKPGDFPWQVLLLGETTAAGALIHDDWVLTAAHAVYGKTEAMSSLDIRMGILKRLSLIYTQAWPEAVFIHEGYTHGAGFDNDIALIKLKNKVTINRNIMPICLPRKEAASLMKTDFVGTVAGWGLTQKGFLARNLMFVDIPIVDHQKCATAYTKQPYPGAKVTVNMLCAGLDRGGKDSCRGDSGGALVFLDNETQRWFVGGIVSWGSINCGGSEQYGVYTKVTNYIPWIENIINNF

SEQ ID NO: 55 - protein, 670 aa, Rat
TLLGSKWPEPVFGRLVSLAFPEKYGNHQDRSWTLTAPPGFRLRLYFTHFNLELSYRCEYDFVKLTSGTKVLATLCGQESTDTERAPGNDTFYSLGPSLKVTFHSDYSNEKPFTGFEAFYAAEDVDECRTSLGDSVPCDHYCHNYLGGYYCSCRVGYILHQNKHTCSALCSGQVFTGRSGFLSSPEYPQPYPKLSSCAYNIRLEEGFSITLDFVESFDVEMHPEAQCPYDSLKIQTDKREYGPFCGKTLPPRIETDSNKVTITFTTDESGNHTGWKIHYTSTAQPCPDPTAPPNGHISPVQATYVLKDSFSVFCKTGFELLQGSVPLKSFTAVCQKDGSWDRPIPECSIIDCGPPDDLPNGHVDYITGPEVTTYKAVIQYSCEETFYTMSSNGKYVCEADGFWTSSKGEKSLPVCKPVCGLSTHTSGGRIIGGQPAKPGDFPWQVLLLGETTAAGALIHDDWVLTAAHAVYGKTEAMSSLDIRMGILKRLSLIYTQAWPEAVFIHEGYTHGAGFDNDIALIKLKNKVTINRNIMPICLPRKEAASLMKTDFVGTVAGWGLTQKGFLARNLMFVDIPIVDHQKCATAYTKQPYPGAKVTVNMLCAGLDRGGKDSCRGDSGGALVFLDNETQRWFVGGIVSWGSINCGGSEQYGVYTKVTNYIPWIENIINNF

SEQ ID NO: 56 - DNA, 28 bp, Artificial Sequence
  Homo Sapiens
atgaggctgctgaccctcctgggccttc

SEQ ID NO: 57 - DNA, 23 bp, Artificial Sequence
  Homo Sapiens
gtgcccctcctgcgtcacctctg

SEQ ID NO: 58 - DNA, 23 bp, Artificial Sequence
  Homo Sapiens
cagaggtgacgcaggaggggcac

SEQ ID NO: 59 - DNA, 27 bp, Artificial Sequence
  Homo Sapiens
ttaaaatcactaattatgttctcgatc

SEQ ID NO: 60 - DNA, 22 bp, Artificial Sequence
  Murine
atgaggctactcatcttcctgg

SEQ ID NO: 61 - DNA, 23 bp, Artificial Sequence
  Murine
ctgcagaggtgacgcaggggggg

SEQ ID NO: 62 - DNA, 23 bp, Artificial Sequence
  Murine
ccccccctgcgtcacctctgcag

SEQ ID NO: 63 - DNA, 29 bp, Artificial Sequence
  Murine
ttagaaattacttattatgttctcaatcc

SEQ ID NO: 64 - DNA, 29 bp, Artificial Sequence
  Rat
gaggtgacgcaggaggggcattagtgttt

SEQ ID NO: 65 - DNA, 37 bp, Artificial Sequence
  Rat
ctagaaacactaatgcccctcctgcgtcacctctgca

SEQ ID NO: 66 - DNA, 354 bp, Artificial sequence
  Synthetic
caggtcaccttgaaggagtctggtcctgtgctggtgaaacccacagagaccctcacgctgacctgcaccgtctctgggttctcactcagcaggggtaaaatgggtgtgagctggatccgtcagcccccagggaaggccctggagtggcttgcacacattttttcgagtgacgaaaaatcctacaggacatcgctgaagagcaggctcaccatctccaaggacacctccaaaaaccaggtggtccttacaatgaccaacatggaccctgtggacacagccacgtattactgtgcacggatacgacgtggaggaattgactactggggccagggaaccctggtcactgtctcctca

SEQ ID NO: 67 - protein, 118 aa, Artificial sequence
  Synthetic
QVTLKESGPVLVKPTETLTLTCTVSGFSLSRGKMGVSWIRQPPGKALEWLAHIFSSDEKSYRTSLKSRLTISKDTSKNQVVLTMTNMDPVDTATYYCARIRRGGIDYWGQGTLVTVSS

SEQ ID NO: 68 - protein, 121 aa, Artificial sequence
  Synthetic
QVQLQQSGPGLVKPSQTLSLTCAISGDSVSSTSAAWNWIRQSPSRGLEWLGRTYYRSKWYNDYAVSVKSRITINPDTSKNQFSLQLNSVTPEDTAVYYCARDPFGVPFDIWGQGTMVTVSS

SEQ ID NO: 69 - DNA, 318 bp, Artificial sequence
  Synthetic
  misc_feature (246)..(246): n is a, c, g, or t
cagccagtgctgactcagcccccctcactgtccgtgtccccaggacagacagccagcatcacctgctctggagagaaattgggggataaatatgcttactggtatcagcagaagccaggccagtcccctgtgttggtcatgtatcaagataaacagcggccctcagggatccctgagcgattctctggctccaactctgggaacacagccactctgaccatcagcgggacccaggctatggatgangctgactattactgtcaggcgtgggacagcagcactgcggtattcggcggagggaccaagctgaccgtccta

SEQ ID NO: 70 - protein, 106 aa, Artificial sequence
  Synthetic
QPVLTQPPSLSVSPGQTASITCSGEKLGDKYAYWYQQKPGQSPVLVMYQDKQRPSGIPERFSGSNSGNTATLTISGTQAMDEADYYCQAWDSSTAVFGGGTKLTVL

SEQ ID NO: 71 - protein, 120 aa, Artificial sequence
  Synthetic
SYELIQPPSVSVAPGQTATITCAGDNLGKKRVHWYQQRPGQAPVLVIYDDSDRPSGIPDRFSASNSGNTATLTITRGEAGDEADYYCQVWDIATDHVVFGGGTKLTVLAAAGSEQKLISE